European Patent Specification EP 3 493 823 B1, published December 25, 2024. Title: Postbiotic-based composition for treatment of ocular inflammation. Applicant: ISTITUTO EUROPEO DI ONCOLOGIA S.r.l. The sequence listing filed with the application follows.

SEQUENCE LISTING (18 sequences)

SEQ ID NO: 1 - DNA, 165 bp, Lactobacillus casei and Lactobacillus paracasei
atgaatcaaaaagctttgaatcaatttcctgaacttacctacacagaacaagtgtcggttgttggcggcgatttgtcagtcgaagtcatcatgaaaggtatcttcaccggtatctttgatgctgggtaccaagtgggtcagtcaatcgcaaaatgggttaagtaa

SEQ ID NO: 2 - DNA, 165 bp, Lactobacillus casei and Lactobacillus paracasei; identical to SEQ ID NO: 1

SEQ ID NO: 3 - DNA, 462 bp, Lactobacillus casei and Lactobacillus paracasei
atgcccaaaagggtcgatcaacatatacgttcacgccttaaaggctttactttaattgaagtggtggtcagcctgattttacttgcggcggtcatgctgttatggcgaccggttttattgcatgtcacgcggttcacgcttcaagaccatgtgctaatcacgtcattgcaagcagagcatgacttgcaaatgtttgtacgagataaaaagttgcggtctgtggccttaatgtcggtaagggtgagaagtcccgagaaagcttacacgatcaatttttatcagaccaaacattttcgcggtatggttcgtgtgatgggatctgaaaatgggcatatgccattatttacgcatctaaccggtgtcaattttagcaaggtagctcaaggctttcgctatcgtctgtatttgacgacttcgcagaagattgacggtggggtgcaaatcgatgaagatacgcggtag

SEQ ID NO: 4 - DNA, 507 bp, Lactobacillus casei and Lactobacillus paracasei
atggccgctgatttcacccaattacaacaagccattcgcttgctcaatgcccatactcgagctgctgatgagcaagcgtggcaagtgctttttgatcgttggctggcaactttatcctctgaaactcgccggcaaatgcaaacagttcggtttaatcatgcccaattgacgttactcacaacgctggatcaaagcagtcgcaaacaactgcgcaatcaggatttaaccgctgctgttccgttctcacaaggcctagtctcacgctatgttgctcgccttgttcaattaaacttgctgacaaaattatccttgcccgacaatcgcaaggcctacattgttgcactaactccgcttggtcaacaagtcgctgccttacatcagcaaatgcatcatcacacaaatgctcaactcgcctctgtacttcatacccttgatccacaagatgttcaaactaccattcaggtactcacaaaactgacggctcagcctttacatcccaagtcttag

SEQ ID NO: 5 - DNA, 261 bp, Lactobacillus casei and Lactobacillus paracasei
atgggcggtgtcatttgttacgcggtgccggtcttttggaaaagaatacttcgcagacacctgattcacgagattaagaccctgaatcaaggattgcagttatcaagcaaagccatgagccaattaattgatccggaaaatccttatatggtatttgctgatgaaaatggtgaactggatttttcatttttgtggctaggcaacttgcgtcaattgaggcgtgaactgcgtctaattaaagaacagaaagctagggtttga

SEQ ID NO: 6 - DNA, 1077 bp, Lactobacillus paracasei
atgagtaaatataaagttattatttggggattaggaaacgttggtcgttccgcagtgagaatgatcgcggaaagacaaaatatttttgaattggttgcagccgttgacgttgatccaaagaagttaggtaaggatgccggagaagtctttgattttgacaaagtcggcgtcaaagtttcagatgatattgatgcagccttgaaacttccagctgacattgtgctcgacttttgcccaacggaaatggacaaacaaggaacattcatgccttctgctattcgactcgccaaatcgctcgatgccggtaaaaacgttattaccacgattccggtatatcatgttcaagacagtcagccagaagtatatgaatatctaaatgaacatgctaaagcacataatgttgcttttgtaccatttggacttttgccaggcgattatgcctcatatatcccactagttttggccggggccatgggccacgtggataaaattgttgttcaatccggtgaagatgactggcacaacacatcaggctgggtcgatgtcttctcatatggcggcgatatcaataaatatccaaaaccagactcagacgaagatctcttggctaagttcatttatgcttattattcatccggcgtatacgagatggccgataggatcggtctgaaatatgataccttcaaaccagagcatgaagtcttcactgcacccaaagatttggaaacgatcaagggtacagtcaaaaagggcagcatttatgcccacagatttaccatggcactttacaacggcaacgaacaagtagccgccttaagatatgttcataaagttgataataaagagacaccagaattaccgatcaataatacgattcatattgaaggcttgccgtcagtcgatgcgcagatcgatggattgatcccagaaagagaaggctacgtttcatcagccgctccagcagtcaacttgatccctagcattctcgagaccgacaagacaggttatgttgaagtctgcgaccttccagtagtgattgccaggccattggatattggcgcaaaaaaattagtctag

SEQ ID NO: 7 - DNA, 561 bp, Lactobacillus paracasei
atggcaacctattcgcagatagaactagacataatcaaatcatttaaagggctgatgaaagaccatgaattcactgagatctcaattaaaatgatcgctgaaaaagccgatatcactcgacgcggcttttacaatcacttcttagataaatatgatcttgtcagtaccatctttgagcatgatctttttccaacagtcatcagtttgacgaatatcaatgactgggatcaagggtcgctgtttatcgtgaattatctccaagacaatcgcgactactataaaaaattgttgtcgcttgaaggacaaaactgtttacagacagacttttataaattgactgagatgcagattgggatcttgatcccagaaatattggtcggtaggaaaatttctgacgaagatcaggcatttttaagcgattattattttcacgcttatatgggactgactaccgaatgggtcaaaggtaaatatggtttttcaactcaggagttcgttaaacggtggaaagccttactcaataattcaatgcataattatctggacaactacgctcgatga

SEQ ID NO: 8 - DNA, 1077 bp, Lactobacillus paracasei; identical to SEQ ID NO: 6

SEQ ID NO: 9 - DNA, 429 bp, Lactobacillus paracasei
aaaaacggcttagaacgctcatatttgcgttctaagccgtttttatcagcataggttcttgacaccaataaacatctttagtaattgatcaaatttaggcaatgtgcttttgtcggtgaatggcgatagccctaccgaagcttcagctgaggttcttctgagccacgcaagcgaagcgcgctagggcaagccaacggcgcgcaggcgaagccggagttaaatgtggcgcagccacacctttttagggagcaacgcgaccagaattttgtatggggtttgggaagaggttctccccaaggtcttttgtggttattaacaagcaaaacacaaacacaagcctcgcgcgcgttatatatacttctaaatacttttaaatactttaagtacttagggagacgagaatggctcaaccacgcgtttaaatcgact

SEQ ID NO: 10 - DNA, 241 bp, Lactobacillus paracasei
acgacctctcgaccacccactgcctcaccaatccccaggtgaaccgggccaagggcactaccgagcaacccgacccctatatcccggtgggcgtggtgaagcagaccgatgggggcatcgtggtgcggggcgcgcggatgctctccacgctgcccacggcggatgagcttttagtcttccccagcactttgctcaaagaagggccgggagccgacaagtacgccgtggccttcgccatccc

SEQ ID NO: 11 - DNA, 7384 bp, Lactobacillus paracasei
attgatcgcctccgggtcacttatatgtaactaataatactcccttctctctttagttacaatagggtacagcctatcgaatcacttacgcttccactttgagataacttttcgttattatttatcaacggcattaacgatatcattaactgtttgcaatgcatcgctcagtacactaattggtgcttgttcaatatactgcatgtgtcgttgtacaaaatcaaaggtgtgaaattgtaacggattcacgtacccttctattttttcagtctgaatcggtaccatcaagcctgtttcagctaagcgattatgtttggcatgcgtgatcggacaaaccaacgctaatccagtcattttggcatattgttgattgctaataacgagcgctggtcgtcttttttgaatttcatgaccccgacttggcatgaaatcaatactcacaacatcacctttgcgtggttgataatgcctagtcccactcacttggtaatacctcgttttctaacgtaatatcttgttggtgtacttgttgcttgtaccaatcaccttcaaatggattgcggtgcttcggcagataaagaatgccaccatcatcacgttgctcaactgtaaattcagttccatcggcgattttaatactctttggaatggttaatgtaatggaattgccaacccttcttgctttaactgtcattgaaatcatcctttcgtatacaccgagtatacaccagcgcgaatgaatctgcaactcttgtgccctcttgtgtacaaacaccactgtcaatttacttttgcctattgtgctttatctcttctcgttctgtcattagtatgccaccaacacggccgacttcatccggctcacctttgatgacgccttgaataccatcgatttgcttccaagtctttacttccaagttcttcaaagactttgatatcgtttttcgatgccggcaaacacttcttcattctgatgcctttcaaagaattcctctagatcattcatcagagattctcctcacttaaacctagttggcgtcaaattccatctcagcaatcgaatcttctaggctgtccattacttcgtatgtttcaatgaagttaacccagctgtcatatggatgtagtttgctttctttaatgctagttctaagcttttcgtacacgttgtcaataaactgctcaaccatcctattaaccgcactattaataaccgcttcgttccactgcttagatgctgcacgctttcgattttgactatgctgatgggacagcgcccggcttctgaacaacgctactgccctgctgttagcattcagataggtttcaaattcttcacgatccattacgtttcctcctcaaaataagcctcatttcatagcacagcttcagcaaaaggcatgtcatcctacatgccttttttctgttgctcttcaatatcagtataaaacgtcctgccgctttaggcaaacgtatgttcgctattaagaacatacgtttgtataataactataaaagatttaaaggaggtcaatcgtatggaaaacaatgtcccgcgtgaaaaatggctttaccctgaccgctgcatgaagaaatggctgggctggattctaagcgaccattccgcctatatggaagaagcggctatctcagaacaaccggtgctcccaaagcctgaacagacacaagaaaccattaatggcgtactcgaagatgcttggcaaaactcaaaaattgtcgcagttcaaatcggtacgccatacgatgatcttctgttaccggatattgaaggcgccgtgattggtcattgggacgctcaggtttatctacagcttaaaactggtgagatgcaatccattaatgcagcggacattcgcaatgtgcaactgctcaatccagatcggtggtgggcgttagtatgacgacaccattagatgatccaacaaggttaccggtacacgacattatgtgcattgactgtaagtccttttacgcctcagttgaagctatcagacgcgggattcatccgttagccgccgacattgctgttctcagcaaaggtaattctcctggcggtttggtgctggctgctagtcccaactgcaaaaagcgttaccacgtaggactgagtacacgccgttttcagctaagggacgatatgtaggtagaacttgctgaaccgcggatggctaattacattcgcaagaattacggtatcaatcgtatttaccgtcagtttactgacgatgctcactggtctccctattccgttgacgagtcctttattgacgttacccacccccacaatctcttcggttctaatgaagaaattgctacccaaatacagaagaaggtgtttgatcagtttggcattgtcacaacagttggcattgggcaaaatcccctattggcaaaattagccctagataacgaggctaagaagtcaacgccttggcaagccacttggacttacgatcgtgtgccagaaacaatatggaaacttgatgacttggttgatttttggtcgattggtaatcgaactgccaagaagcttaacgcgattggccttcataatctttacgacttggctcatgcagaccgcgccattctgcaccaaagattcggtgttctcggtgatgccatgtactttcacgcatggggtattgattactcagacttaacccgccgctacttaccacgggccgaaaataaaggctacggcaatagtcaggtactcatgcgtgattacactcaggcaagggagattgaagtcatgcttagcgagattgctgatcaagtggctggccgaattcgccatcaccaagtccaaggtgaggtcattagcgttggcattggttatgctgatgcagaagaagctggcacctccggtttcggtgcgcaaatgaagattgatcccacaaatcgcacagacgatttaattcgcgctactcgatttctcttccatagtaagtggaacggacacgctgttagaaatgtctcagttcgcgttaatcgcatcagccaagcaagtacaatgcaacttagtctatttgaatcagcagagaaggaggaagcaaacgcggctcctatgctgtaattacggataaaagaatcaccatcattaggtttttcgtctaacaattttaggaaacttcactttctaggtcgtaactttatttttgcaatctagggttttttaaatatatacattttagctcgtttgtgtttaatattataatcacaactataccaatgataaatgtctaacataaatatacaaacatgttgacagaagctcttgaatacgtttacaattatttcgttcaggcgagctttgtttttgaaaaagtattaatacaagataactaggttagtggctgttgaattaggcccccgatttcgggaccacgacagtcacttgatactcgatttttatcgtttgctggcttgatcgtacattgaacgaaattggtacagaaaaaagagctaagagccgctccaaattagccaaaacgattgcggcgtcaatgcttacggcgatcgtttctgcagttttagctgttaccagatcaagtcctagtttccctttgatgaaggcaaactcacgctcgatctcacctcgtcgattttcggcttgtcggtctgccttacgtttggccggatcgacctgcttcggccgacggcccaatctaggaccgctaagtttgatcccaagatctgcgcacagcccgatattcgcccgagtccgataaagcgtatcagccaagatctcatccgggtatgtaccatacgtgtcaaaataatggtcgatcgttgctggtaagtcagcactttcgttaaacgcattgaacgcaaaccgttcaacggccacgacgccatgactgatcgatacgtcgatcttgggcccgaattcgaccggatcctttgctttgccgcgaatgatcggtcggatcgctggttgatcaaggcttacgatccgatccgcgactcggtgagtgtgctgtcgatacatttcagtttgttgctcatacaattttcgaatgatcgttaatcgttgtgtctgccgttgattcaattgcccgccttgtgcttgcagttctttgacgtaacgcaagtcacgtcggatgtactgtaattgagccttgatctgcttatgggtcgttttcacccaacggcggggtttacgtgaaaaggcggtccacgtttggtgggccttgcgcttataggtacgcggcggtttgaccgctaattgcttggccatggctgcgatgaatcgctctaaattgagccgcgcctgattgagtagctgcgtatcctgcggatacttgatctttactgggaccgcagtcgcatcagtgatcaagatcttctgatggccaagtttagcttggaggcgatcgcggacaaaatcgctaatgatgttcgtgatcaactcggaaagcggcgcgatccggcgcctgaaataggacagcaccgaaaatgaaaacggtgcttgcggctgatactctggcaggccaataaaatactgataagccggtgtatcgcggatcgctgcgactaactcacggtccgatagctgagtgcgctgcttgatcagttgggcgccataaagcagccgaaagggtttacctgcccatcctaagttagacgggaaagccaattggtacgcctcttctagttgcggccacggaacttggtcggccagttggacccactcgttatctggacttaatggggtgcttaagccgctaccaaacgatttgatcgataattgaacggcttttcgacgataaaccatgatccatgcctccgatagggtcgtgtcaaatgcaaacgaaatgagcacgatccgtaaattcatatgcattcattatacgacgataacgggttcaactcgcatcaaatgtggttatatcaaattattcaacagccactaggttaagatcttcatttaagtgatattcatttgcaagcaattgaaaattactcatcacgaagaggatttcattggccatattggatagcacgcaaatcacttgctttaagaaaatcagttcctttaatgagtctcttaaaggacggggctctcacttgtactcacaatcaatgttaactggagatcaacaatatggtcatagattcccataataacattgacttgactatctaaaagaggcttctaactttgatattggtggggttattggttgcttggctgtaagcagataatcttaacttgggttattttcattgtgttgtaaagacatttgttataaaggccgaagttatcgctttgacttgtaataaattatttttgattgagatatcagaaaataaacgggggataataatgaaaaagattattaggattgttctttgtgttgttagttgcgttagtatcatggtcggatcgcttgggttctattcaactccaaagatcgttaaagccgacagtacatctgttacggatgtcgacattaatacctatatttctagcatgacacttgatcaaaaaattggacaaatgtttgtagcacgaacctcacaagatactgataaagctcgtgctgatatagcaaaatataatcttggcgggctgattgtttatggtgttgatttcactagtgttaaagggacaacagctacagaagctcagaataacttcaagatgaagatgcaaggctttcaaaactcggcaagtctgccactattgattggtgttgatcaagaaggaggggcagtctcacgcttatcacaaaatcctctaattgccaacggcagaagttttccttcaccacaaatggcttatgctaatggtggaatgaccaatgtaacaaaagaagctagtgaagtcggaactattctaaaaaatctgggcattaactggaactatgcaccagttgccgacagtacgcctgacacctctagttttatttatggtagaacctttggtcaagattacttggctactgcaaactatattacgaatgtgatccctgcgtggcaaaatgctggcattgccgcaactctcaagcatttccctggttatggatccgcgattgatacgcatacggattttgcagtcgttacaaagtctaaggaggattttgaaaaagaggacttgcttccctttaagtccggtattacagcaggggcagattctgtaatgattgcacatatagtaatgcaagctgttgacccagtgtatccagcatcattatcacggaaggtcgttaccgatttgttgcgtaatgaacttgggtataatggcttaataattaccgatgcattggaaatgggggccatcaagcaatttgctcaagaacatgatcaagttcctgttgatgttcttgctgttgaagcagggaatgattgcatcatgaataacgattatgaaaccgctattccacagattcatgcagcagtaactaatggaactattaaggaatcagaaatcaatgaacacgttttccgtattcttgatctcaaacgcaaattagggttgttaactaaaggacaacttcagcaaaaaaaagttcaggttgacaatgtttcctacagcagtgacaacaaaaaggcaactgtgagtggaacagttgttgatagtgattggcaagttggagaaccattatcggttaaagactcgactgggaaggtcattattaccgcagacgttggtgccggtggtaagtttactttcgatgttcctactaagtcccaagaacaagtattaactctgactactaatttacccaacatcgctgattctcaaataactattaaggctgtgagttcatcgaatactaacaaagctttgctagaaaacttgatcaacgctgctgaacagttggatagtaatcaatatactgtcaagtcgtgggaagaattacaaactaaactaactgaatcaaaatcgattctgaacaatgatagtgctacacaagatcaagtagacgcttccgttaatgctctacaaattgcccttaagcaattagttcctgtatcaaatagcggaaataatggtcaaagctctaatgatagcagtaaccaaagttcatctagcagtagtggcaaagaatcatccagcaatagcaatgccaatattactagtaaggatcagtcagctaaggattcaaatacgaggcctaaagaccatagtcttttgccaagtacaggtgaacgggtgatgacgggaatttctgttctaggggtaattttaatagcttgtgtgactatattatatattcggaaaaaaggacgcagcttttaattagtctctgcgtcaactggcgttaaaaactagattgaagtaataaagttaccacctggaaagaggcatgctcattgcttgcaagggtgtcgacgtgtaatagaaaagttgggg

SEQ ID NO: 12 - DNA, 1410 bp, Lactobacillus paracasei
tggcgtgggcaacgtgcacgttttctagtcgctaaactgtgaacaatgctcgtgctaaatgcaaaactgagcaaggagatgaactataagcgggggaccctttgctattgaggaggaaggcgaagtagagaaagagcggtgatttgaactcgaaacagcggcgccgcaggctagcagcactgttagattaatcgccagcagcagatactagacagcttcttaaaggcttgataatagcgttgcgccatttcaatggaactagtggtcaaaatcgcattgtagttgccatgacccaaactcgttttacgcgggcctttttgtaaaatatattgaacaacttggttaatatgttcatcggtctcaaagtcagccggagttaaatacgtttcttccaagtccttcactgacatcgcttgaatcttggcttgaattttcgcttcatcagccgtactcagcaggcggccttgcttatcacgacgagctttaacgcgctgagtttctttttcaagggcccgggttattaaagcgtctttaccaatcgttgtcacgtgttccacattaaatggtaacactgcttggtcctctaaggcgtctcgcaagttataaacatgacagactttaccaaatagctcctccgtcgtaactgctagatcacctttgagctgtttcttattttcattaaaaatgggggtgccagtgtaaccataccagttactattgataaacgctgctcgaatttccttttgcatcttaccaaactgcgaccggtggacttcttcaacaaagaagatcacccgttgctttaaagtcttactaaagcgggattgcttaccggttgccagctggacttgcgtttttttgaccgcccgatggagcttttgaatcgaggtgaccaagaccttaccgtcattttgttgcaatttacgcattaaatcaccggtgttttgggcttcgttaatggcaatatcatcattggcagcataggcactaaagttgctggttgtctgttcgtctaaatcccgccggtcaactaagaagatgaccttatcgacaccaggatcttgcgcagctaatttagcggttttatatgaggtgagtgttttaccagaacccgtggtatgccaaacgaaaccatcctgatggtcatgaatccggtgcatcacggcttcaatcgcataaatctggtaaggccgtaagagaattaagctttgccgctcttggtcgatgactgtatattcactgaccattttgtgggccatgggaatattaaggacttggcgcgtgaacgctaacccgttttccacggggtgattatcccgcgtccgccaattgaacaaaaaggctttattgaaatgatccggttcggcattcgcaaaatacgccgtactatccggcgtcataatcacaaac

SEQ ID NO: 13 - DNA, 592 bp, Lactobacillus paracasei
cgatctaaaagctaagttattttccaagatatcaaacaacttcttaacccaagaatcttccacacataggacaataatgaatccaaatagattcagctttttcctgcaaaccgggatcagtataaacgtccagtaccggataatcacgcattaagttcagctgccaatgggtatcatctaaattaaaaagatccgatttagtgtctccccttactacattatggcaatacacacaactgttgttatacatgcttccttgctttttgattttaaactcctccattttgcatattataagaagattacttctacttgatatatagatgctttccttgcgagggtaagtcagacaaggaagcatttctaacttgagatacttaagcttgtctcaatagatgtagatagcggctccccaatcggatattaacagctcaactagtcaaaccagatatataaatgtgacacaagctggaatatatatcattatctagataattcaaattgagctaataaaatcaataaagaaaattttaaataacattattttataaacccctttaggattttcccgatttgatattctacgtatgtt

SEQ ID NO: 14 - DNA, 2233 bp, Lactobacillus paracasei
gagtatccaaaaatacgacgggtatttgaataggatacttattaagcgagaatggtattggaaatctgtggcagccactcagcggaaccatacctttatcccaaccccacgcaaaaaaaacatcaagtaatccgtcagatatgatgacttaattgtgggacagttctaatatgaagaaaacaggttagataattggggtgaaaagatggcaacctattcgcagatagaactagacataatcaaatcatttaaagggctgatgaaagaccatgaattcactgagatctcaattaaaatgatcgctgaaaaagccgatatcactcgacgcggcttttacaatcacttcttagataaatatgatcttgtcagtaccatctttgagcatgatctttttccaacagtcatcagtttgacgaatatcaatgactgggatcaagggtcgctgtttatcgtgaattatctccaagacaatcgcgactactataaaaaattgttgtcgcttgaaggacaaaactgtttacagacagacttttataaattgactgagatgcagattgggatcttgatcccagaaatattggtcggtaggaaaatttctgacgaagatcaggcatttttaagcgattattattttcacgcttatatgggactgactaccgaatgggtcaaaggtaaatatggtttttcaactcaggagttcgttaaacggtggaaagccttactcaataattcaatgcataattatctggacaactacgctcgatgaattacacagattggattaaatgagaaagatgttacatttgtgccaatatgtgaattgataaatatttcacaaggaactattctttccctgtaaacgaaagttgacttgaaaggagttagttctgatgagtaaatataaagttattatttggggattaggaaacgttggtcgttccgcagtgagaatgatcgcggaaagacaaaatatttttgaattggttgcagccgttgacgttgatccaaagaagttaggtaaggatgccggagaagtctttgattttgacaaagtcggcgtcaaagtttcagatgatattgatgcagccttgaaacttccagctgacattgtgctcgacttttgcccaacggaaatggacaaacaaggaacattcatgccttctgctattcgactcgccaaatcgctcgatgccggtaaaaacgttattaccacgattccggtatatcatgttcaagacagtcagccagaagtatatgaatatctaaatgaacatgctaaagcacataatgttgcttttgtaccatttggacttttgccaggcgattatgcctcatatatcccactagttttggccggggccatgggccacgtggataaaattgttgttcaatccggtgaagatgactggcacaacacatcaggctgggtcgatgtcttctcatatggcggcgatatcaataaatatccaaaaccagactcagacgaagatctcttggctaagttcatttatgcttattattcatccggcgtatacgagatggccgataggatcggtctgaaatatgataccttcaaaccagagcatgaagtcttcactgcacccaaagatttggaaacgatcaagggtacagtcaaaaagggcagcatttatgcccacagatttaccatggcactttacaacggcaacgaacaagtagccgccttaagatatgttcataaagttgataataaagagacaccagaattaccgatcaataatacgattcatattgaaggcttgccgtcagtcgatgcgcagatcgatggattgatcccagaaagagaaggctacgtttcatcagccgctccagcagtcaacttgatccctagcattctcgagaccgacaagacaggttatgttgaagtctgcgaccttccagtagtgattgccaggccattggatattggcgcaaaaaaattagtctagactaggctttcgaagctgctttgaccattaaggttggagtagctttttcatttgcaagtaaatcattacggcttgtgtatacggtatacaaaatggagaaaacgctgactagtttataaatcattgagacttaacggccggataaatgctgatctgattatagaaataacaacaaaaaggccacgctaaaaatcatattaattataatcgggaaatttattaataatattcaagaaaaataaaaaccgtgggtacattatttaaaa

SEQ ID NO: 15 - DNA, 5866 bp, Lactobacillus paracasei
tttgaaactaagacgaaagctgccatgtcaaacaaagccgccataaatgccactgtcacagatccatcagccgcaatgccagcatcttgctgaagttctttaacagcattaagggtgttattcgtgaactcattattaaagtctactggactaatccctttgcaccagaaagccccttgaatgagttgagcaatgttccccttatatcctggcttcagactacctacaacaggtgctaaggcgtttttggtcgtctcgccaaagccttcaccaatagcactaataccgatttcgtgctgtaatcccattcttaggctataaattgttggccatcccgtttgcccgttttctggagctgcgacaaagccaggaacgctaccatacgttttgttgagccatttttgaacggctcgtactgcttcatctgccattttaaagtctccttttttgttttagacagcacgtctgccgtcacaaaaagcaaacatatgttcggattcatttcatctcttcaaagcttcgaaaggcaaccctgatccacaaataatccttttattttgaacttagcaaaaaaatgaggccctcacatagtgttgaagttgcctcattcttaatgtctatatttaaagtattgccacaacgatggatcatcgaacgctcatggacttggttagacatgtatcgacgactatgaaaatgtgggcgcaagctcaatttcaccttccaaatgtttgtgctatctcatttagcgctggtttttttaggatagactagacaaggactaataatttctcaagaatcccgcaactccactattcattcgtcgaaatccccactgatactcttgtccttgcacgttcgaccaagcaagaatgtttattccgataaccgaattgttgccatcaagtaatggacctcccgacatgccatgatacgaattaatttgttgtgaaatatatattcctagtgggtcctctgaaaagggtgtgacagtcccacttgattgaaccatgactccttgaagttcgtaccctgattgcggatcgccagggaatccaatggatcttgctgccatcgtatcagcagggttcgtatttaaattaagacccgcaggcatactaccagacttcatagagacaattgcagccccgtaatcattcgaagtagctgttgaattattaatccatgcctgtggcactatcaatctattcaatactccgtaaccgaccccttgatgatttgcttgactatcaccaaagttaataattcctccagaaatataatgaccatcatataacatgtgtgctgctgtccctatacggtctactccaatgctaaatccagtaccgccagaagttccactgctcagctctgtgccatttgagttagagatgatttttttatacgaactgtcaaggtatggtgagttaatgaccatgacaccatttgccatcgaaaaccacgtgctcaaaaccccaacggaactgtacggcgccgaattggggtttgacacaggtgataccgtcctcacagatagatgattagacgatttattcagtttcgcaagatattcggacgtaattccttgaactttctttccttcttttaaatcctgatattgatcaggtgtataagctttgacactccctttaaaatcgggataagaatactgatattgtcgaatgatttcattcaaaaactgttgtgttgtcgtctggttagtcaaaacaatatcattctttggtaaaacatggctattcgctgccaaaggatttgccatactatcagcacttacacttaccgtttgaacttgaattatcgctaaggctgcagctatcatagtgatatatgcccatacttttcgcaatttaattccccctttttcttaaaatgaaaccgcattcacggaggcttgtcaatgcttttaaaaaacaaacgttacttttggctcatcttggctgtcagcataattggagtaattgttcttgcggtgttatggcgcatgaaccctgaaggaacggcctcaaataagtttgaacgtcccaccattactattaaaaaagtcaaacttattaagcacagtaacagtattgctgtcacatttgctacctctccaaaaagcaaatatacgataagtgatcttaaagagaatcaactttcttctggcatttcgaataaaagagaaaataccgtttcggaattaaagccctcctcctctaagcttgcaatacgggttaagcataacaataatatacaaaccaaagtggtttctgttcccattggttatcatattatgaaaagtgccatttcaagaaagccaattcctatgggagaagagtttaagtacaatggaaagtcgcatgttttatttagcatgaccattacccctaaaaaacaaaacaagaacagtataaaaaacaccactgcttttaacataacggttaaaaatgatcactaccttgtccctgtcgtattagataccaaataccttactgtttctgattcagaaggtaactcattaaaagtaaagccattctcaaaaatttctattccagcaaaaaagaaaaagaccattgcaataactattgagggcgttcccgcaagctctgccaatggtctagttataacgtataatactgtcgatttagacttaccaatctcctttataaattcctgaaattacactaactgtcccccaccttgacagtcagtacactcaaactgtctcttatgcttacaaacacgtaatttaggcggtttttaagcaaaagtcgttagttttcataaatgttatcttatactctaatgagatctagcttgtgataataaggctgtttttctttgacagccttattaagcacactaatcaatgtcaattcgaagtttttggtttcctacttggccaactttgttatcagaaattccaaaactcattgcctcccgccaccatatatttatcgagccattttgaaaatgaaaaatcgaaatatcggtctgcttctattccgggatgagttagatatgattttcctaaccgatacttctctatatcaatatacatatctccgacatcccttatatggagaatgggtactttatttacaaaacttttaggcagtgcctctttttctttaatcatttttctaattgaatagacttcacacgtatatcccataggaatcccttcgattgttgtgtcaaataaaaatagtccattagtaatcgagagaaactcaatgtaatcctgtggaaggttccacctttttattttttctatatcatcagcgtgtgcaggaggttctatcttaaaagaaacattttgcacatctccatctaattggaatgttgagagcgctttttccccatttttcgtcacctttattaaagaattaattcttcgccgaattagagattccaaatgagttcctcctcaatagttgttaaaccacgcggtgatcaaccgatgatttggtgttaacaccggcatcaaattattaaagtcatttgttccgccataaactctcgggcgaatatgatgcacttctcgagaactccaaaaatctgcagattgattgccatatgtttcactgaacgttttaatataaatatatctatcttttgatgaccaactaggagattttgataacttagtccaggtagtattaataggtgtttctgcatcttttttagacacgggatcaacatattcagggaaattctgtcctattttattttgtaaatagatggccgttggtgggattggttttacattagccgctccattaactcctataaatccaacagcgccagcaacgttaaaaaatgtggttttggctggcaattctgtaaaaccaagtaatcctgtttgcaaaccgcctattttgctaatgggtgccagcgtattggcattcaccggacctgcaagggtaggctcagtattaaattcaatttgcacatcaactgcggctggcgggacaccctcaatagaatcaatccagaaattgactctgaattttccggatatgtattcttccgataagtgccaggtaatatttgtaacaggaacttctgcacgagaacttatgccattgccatgactattattcagtaccacttgttttccagaagcgataattggttgtccattttctggattacttcttgataacttgtcagcattggtcagttgagtattgttatcgctaatacggctttcagttgaaacaatttgatttaaagattgtgttgtgtctgcggatacaattgttgaatacccaagcaaattgactagaaagagcccgaatattagcccaataactttccactttttcacgcctattatcttctttccaaagttcttcagtgcctggcaataactgtatacattgagcagtatagtcgctattttatagctgaacaactcataaagctcaattattattagcctataaaaccactgcctaagtgaattgatctagaacgaagcacgccgaagaagtcgctaaatgtgctaagaaaaatgtgcttgaatagctcaaaagtaattagcgtctccattgaaaatccgttatttttaagtgatctagtgttaactatgaatcccaaataaaaagcaaaatccgtaaatgccaaattttcctttttgacgtttttctactgtcgcgagatttgcaagtgtacgtacacttacgatgaattgacagaatctcagctgcgctgatcgtcaattttgtttgggggcacgcccccaatccccctgttattttgaagggaggtgagtcccccttcaaaatcaaaatttaaacagcatctgccgccatcttttcgctgaccttctcacgatgttacacgtggtgttgacacccacttgcatttagagtttcattcaagttgaacattgtgtaatatatgagttgcatttgataaacatatcagttgctatttgtgcaactttaaagcttcggctaattcaacgttctgttaatttacaagcatctcgacagtttctgttaaagcaacatctacgcttcaattcgagcaactcactatacgtatgccgagttgcagacaagctactatatagctgtacgcgctgaaacaccaaaaatcgttcgtttatgcccaataagcgaataatcttgctcaggtgtagtaaaaaactgtttacgtgtagtgaatggcgctagcccttgtcgtaactggcatcatccacgtgtagtaaaacgcgttttactacacgttcgtaattttttcacgtggagtaaatggcgttttactacaccttttgaccccaacgtgctatcacgacaaaccaaaccgcactgcggtttaccccaattttggggtcagttttgccttatgctctttcatgattttaggcgcgttccaagcagtctcaaaaagtggtcgatccaggcgagccgatttttgagaaggattggatagcaactcaatttattttgatcttttgcttggagaaaaacgttcacgttttgaccagggccgtcgcaactgttgaccaaaactcgtccggtaacgtgacgctatttaaacgccgcgttggtttgctagacgaccattcatcatcaccattcaggaggtttttgaaatgacaaagcaagacgaaacacaccgggtcatgttcactttgaccgatcaggcgattgcaaaattgaatcagctggtcgcaaaaaagcaacaggaagtgaatcaaaatccggaactggctaagtaccatgtcagcgtgaccaaatcaaatatcattgaggactggttatcaaagcagtgagtttaaaaagcgctaaagggcctgtactagcgtttcttactctggtgggtataattaatgctctctacatcaaaaacg

SEQ ID NO: 16 - DNA, 11007 bp, Lactobacillus paracasei
gccacgaacctgtagccgtttggatgaagccatataatactggaccaaccgccgcaaataagtagccgacactttgagcaaaatcaggaatactaatctactttgcccttaaaaaatcttgagatgatccatatcttgttttgccttcattactgtagttggtcataagaagtgccctacattcattagattacttgtctaataattgtagggcacttgggttgagaaaaatgatgttaactaagaatgcaaacgaactaaaatctttgcttgctttttatccttttctaaggattcaattccttctgaaactaattcatttaattcaatcttttttgtaatgacctgtttgaatagtgaacgatgggtatctataatcttaattactcgatcgaagatattggcatatccataagatgttaataaactaccaccttttttaagaagagctctaacatctacaactggtggatgttgaaataatgcaatcacggtaaccttgccaccatttttaagagcctgaatggcaccagtaagtgtgggttgtacaccggcgcaatcaaacgcaatatccactccctgattttccgtgatagtgctgatagcgtgagctaatgacttttgactatcagcacgtattgggtattgaattcctaattcatttgctaaattcaaacgttcctctgacatgtcatttattatgacgtgatgtgcaccagaaatttgtgctattaaggccgtgaacaatccaattggaccagcaccttgaattaaaacatcatctccaggagacactcggcttgccataactgcctgtgcagcaactgaaactggttcaactaaggcccctaaatcaagcggaaagctagctggtaagagatgtgcaaaggtactttttacattgcacttttcagctaagccaccgttagccgaaaatcctaagaatcctgctgattgatcactacctatagcatgttcacaccaattataatgaccagaaagacattccggacattttccacaagcaatcattggttcgactgcaactttatctccaattcttaatttagatacttgttttccaattttagaaatcgtcccagaaaattcatgaccaggaattagcggggcttgcatatgggttagcggatgaggtattgtcgccaaatccataccctctaaatattcatgaatgtcactaccgcaaataccattaaatgcaacctcaatttgaacttcatctggtgcgggatcaggaatatttcttttttcaaagcggatatccttaggaccgtaaataacagctgccttcaccatagtcatagtgcttcgcttccttcatgttcaatatagcacaatcgtatataaaatagtgaatagatttcagtaatgaagttaccatcttgacttaacaaaaacttgctaactgattatatgagaaacttttacttgaaacatttttggtgattaccattaattccctcggacatattttgaaaaaccctatttgatgctgattgcaaattattttatgcgtatttattaagggtttctatgttgaagtatatagcaaacttgttcaagtaactgactttcacgtgggctttagccaagagatgctgagcagcgaacccaaggggtgttactcgcccacgcaaaaaagaaatccaattgcattccagtatgagcgagaagcaagccattaagacgctgattcatgaactcgcgcacagtgaattacattgtgatccgaagttaaaattggatcgttcaaccatggaattggaagctgaaagtaccgcgtttatcgtttgtcaacatttgggaattgacacgagtgattatacgtttccttaccttgctgtttggtcgaaagataaggatctttcccagctctccaaaagcttaacgcgtatccaatccaccgtcgaaaaattcaataaaaccgtcgatcaaaaccttgaaaagattcgtgagaaaccgttgacgcttgatcaaaaaatagaacgcgctaaaaccattgcgacaacggaaaacatcgcaaaaaaagagcaagggctggtgcaagcaacgcaggagaaaacacgctaacccatttgttgaatactctcactcaagaggacactccagcccttgatcacccaagaaaggaattaccaacatgaaaaccattgacgaaatgaacgaattcgatcgtgacattatcttacttcaccgcaagtctgtgagcgaagatacaccgcaggcaattcttgtgaaagtgaaacagattcgtaacgcaattgccgacgaaaaggcgggtaaagaagatccaattgagaaagaatttacactcgaatgttacgacgaagcaatcagaaaactaagggacctttcggtcgctgattatcagttgtggttgcgtcaaaacaaagacctggaagggtttgaattttgattttgaagggtgtcgtagaccccttcaaaataacgggggattgggggcgtgcccccaaaacaaaattgactatcagcggagctgatattggatcaatttatcgcaagtggacgtccacttgcaaatctcgcgacagtagaaaaagccccagaaaagcaaatctgaaaaaatgtaacaggcacttgatatcaagtgccttattgtttctaggatcgctaaaaataacaggaggtggttacatgaagcaatctgatgaacaccgcacgcgttcagtgagaagcactgtgcgtatgaccccagaggagcgtgcttgggttgatatgagaagagcctctgtcggcaatccaaagttcaatgcatttgcctgtcgcgcactcacgacgagcaagatcgttcatgtacattttactgatactaaaaagttacttagacagctgtcaagaattgggaataaggctcctatgctgtaattacggacaaaaatagtttgtgcgataattacagcataagggcctctaggtcggagcccaggaggcggagaccgccgcacagcccaaccccacgccgaaccggaggccagcccgcccgcaccgcggccgcaatcatccacccaacgccccccaagtttttgatagcggtaacaacgcctgtgcgcttgtcgtggccggccttttttcataaggttggaggagaaaggaagggtggttatgggcgcttggtatgaacacgcaattatttaccaaatctatccaaaatcgtttcaagacagcaacggcgacggcatcggggacctgaacgggatccggcaacggatcccgtacctgcaagccctcggcatcaacacggtgtggctgaacccgatcttcgtctccccacaggtggataacggctacgatgttgccaattacttcgccgtggacgaaaccatgggtacgatggccgacctggaggcgctgatcgcggctctgcacgcggccggcatccgtctgatcatggactttgtgctaaaccacacctcggatcagcacccgtggttccaggacgccattcacgccaaaaatagtctgtaccgcgactactacattttctctggccacgacgggcagctgccaaacaactggggcagcttcttcggcggatcggtttgggcgccggatccggcgggaaccgggcagtcgtattttcatctgttcgaccggcggatgccggatctgaactgggccaatcccgaggtgcggcgggcgatgggagacgtcgccacgttctggctcggcaagggcatcgacggactgcggctggatgccttcatccacattgccaaggccgatctggggcaggattaccccctggctccggggcagcagacgccggtggtggcggagccgtttttctccaacctcccgaaggtgcaggaatggctgcggccgttctgcgaccggatcaaaaccgactaccccgacgcgtttctgctcggcgaggcggcatcggccaacgttaacctggcggcggattacaccgcgcctagccagcacctgatggacagcgtgatcacgttccgctacttcaccgaggacgaaagcggcctggatccgcggctgccggcgcagtaccagccgcggacgctggatttcccggcgttcaagcaaacccaggcggtgtggcagcagaccctcgccggggtgtcgatgccgacgctgtactggggcaaccacgacatggcccggctggcgacgcgggtggccaaaaccaccacccaggcgcgcagtctggccatgctgatgtacctgcagcgcggcctgccggtgatctactatggcgaggagctcgggctacacaacctgcagttcgatcacgttgatcagtttgcggacgtttcggtggcgccgttcgtggccgcggtcgaggccaccgggcagtcgcggagcgcggcgctggccatggtgtcggcgacgcacaaactgccggcacgggggccgatgccttggacgaccgggttgcaccagggcttttccaatcacctgccgtggctggttgggcgcagcgaggacgtgaccagcgtggccgcgcagcaggccgatgaggccagcatgctgcacttctaccaagcgctgattgccctgaagaagcagccgctgtttcaggccgggcattaccggctgctgacgacggcgccgaacctgtacgtctacgaacgcacgctggccagccggcgggccctggtggcggtggccttggatgagcaaggcgccaccttcaccgtgcctgaaggcctgacgaccgtggcgctggccgccggcgattaccaactcgaaggtcaaacgctcacgcttggcgcgaacgccggcgtggtgttaaacgaaaggggaactcgataaccatgcaacttgcagcattacggcaccgcccagaaagcgaagattgttttttgtacactccagatgagctgcggctgcggctccacacagccaaggccgacgtgcaggcggtcatcgtactgtacggggatccgtatgtcaccgcgccgaacccgaccaccggagaaccggaattcgcctaccaagaggcggcgatgatcaaaaccggcaccggccaaaccagcgactactggaccatcagcctgaccgcgccttatcaccgcctgcagtaccagttcctggtgaccggtcaggacggcaacaccgtcctgctcggcgaccgcggcttgcgggccgacagcgccgccaaccgccgggccgatctgttccgggtgccgtacttccacgccatcgacacggtacagacgccggcctgggtcaaggaaaccgtgtggtaccagatattcccggaacgcttcgccaacggggacaagacgaacgaccccaagggcaccaagccttggcgtccggcggatcacccgggccgtgaggattactacggtggcgacttgcaaggggtgctggaccacctggacgacctgcaggcgctcggcgtgaacgggctgtacttctgcccggtgttcacggcgatgtcgaatcacaagtacgacaccatcgactacttcaacatcgaccctgcgtttggcgacaaggccttgttcgccgatctggtcaaccaagcgcaccgccgcggcatgcgggtgatgctggacgctgtgttcaaccacatgggcagccgcagcatgcagtggcaagacgtgctgaagttcggtccgcagtcgcgcttcgcctcctggttccacatcaaccgttttccggcggcgcccttcgccgcgccggaacagggcggcgtgccgcagtacgacaccttcgccttcgaaccgcacatgccgaagctcgacaccagcaacccggcggtgcaggactacctgcttgaggtggcgacgtactggatcaaacagttcgacatcgacgcctggcggctggatgtggccaacgaggtggaccatcacttctggaaacggttcaatcaggcaaccaaagcgctcaagcccgatttcttcgtgctgggcgaggtctggcactccagccagccgtggcttaacggggatgagttcgatggggtcatgaactacgcgttcaccgagcagatcgaggcccacttcctgaccggcaagctgagtgctcctgagctgacggcggcgctgacggatcagctgatgctgtaccgcgaccaaaccgaccaggcgatgctgaacatgctggactcgcatgacaccgcgcggctgctaacggtggccggcggcgacgaggacctggccctgcaggcgctggccttcaccttcctgcaaaccgggatgccgtgcctgtactatggcacggaaatgggcatggccggagaaaacgatcccgactgccggcggccaatggactgggcccagctgaagggcccgatttggcagcgtgtgcaggcccttgtgaccttccgccgcgcccagtcggcaacgctaggcaccggcaccacggcgctgagcgtgaccgcagccgggctgcttaaggtaacccgcacaggtgagcacaccgtgacggcgtattttaacaccaccaagcagatggcgacactgaccgtcagtccattactggcgcagggttacgccggccagcggctggcgccaaccgggtttgctgttatggttcagtaagattatgttagcggtaacaggcaatttgaccttttaaaagcgttttcatattatcataatcaaaagtgtagaaaagttcaggtggcgcaattcacctcccgaaagtgaaggatgcaagatgaaacggatatttgaaatcgacccgtggctggtgcaaagccaccaattgaaccccaacgagaaacgcctgcaggaaagcatgaccgccatcggcaacggctacatgggtctgcgcggtaacttcgaagaaggttacagcggtgatcacctgcaaggcacgtacctcggcggcgtctggttcccagataaaaccgtcgtcggttggtggaaaaacggctacccggattacttcggcaaggcgatcaacgcgccgagcttcatcggcatggcgctcaccgtgaacggcgagcgcgtcgatctggccaccagcgtctaccgcgatttcaccctcacgcttgacctgcaccagggcctgctgacccggagcttcgtgttcgagggcaaaaaggccacggtgcgcttcaccttcaagcgtttcctcagcaacgtaatcaaggaggcggcgctggtgcagctcaccgccgaaagccttgtcggaccggccgagctgacggtggccgcacagctcgacggcaacgtcacgaacgaggacagcaactacgacgagcgcttctgggcaccgcagggggaaaacgccgcggcaggcaccatccagctgcagaccaagcccaacccgttcggggtcccgcagttcacggtgctgctcaagcaaagcctgcgccaaggggcaacccttttacccggcaccgtgaccaccagcaccggccagctgaccagcacggtcacgctgccgctggcgccaaacgtgccggtccagctggaaaaggacgtcatcgtggtcacgagccgcgacgtcgcccctgaggcccaggccgaagcggccgcggagctgatgacacagctgcagggccaaagctttgcggcccagctggcggcacacaccgccctgtgggccaagcgctgggcccaaagcgacgtggtgattgaaggcgacgacgcggcccagcaggggatccgcttcaacctcgcccagctgttcatgacctattacggcgacgataagcggctcaacgtggggccgaagggtttcaccggcgagaagtacggcggggcgacctactgggacaccgaggcgtacgtggtgccgatgtacgtcgccgccacccctccggccgtgacccgggcactgctgcagtaccggcacgaccagctgcccggcgcctaccacaacgcccagcagcaggggctcaaaggggccttgttcccgatggtgaccttcaacggcatcgagtgccacaatgaatgggaaatcaccttcgaggagctgcaccgtaacgcagcggtcgccttcgcgatttaccagtacacggcctacaccggcgatgaaagctacgtcaaccacgacggcatggaggtgctggtgggcatcagccgcttctgggcggaccgggtccacttctccaagcgcgccggcaagtacatgatccacggcgtcaccgggccgaacgagtacgaaaacaacgtcaacaacaactggtacaccaacacgatggccgcctggtgcctggagtacacgctggcccggctgccgaaggccgatgccgccattcaggccaagctggccgtgagcgccgccgagcagcgccagtggcaggacattatcgaccacatgtactatccggaggacaagaagctgggcatcttcgtccagcacgacaccttcctggataaggacctgcggccggcaagctcgattccggccgaccagcggccaatcaaccagcactggtcctgggaccgaatcctgcggtcgccgttcatcaagcaggcggatgtgctccagggcctgtacttcctgaacaatcgcttcacccgcgagcagaaggaacgcaattttgacttctacgagccgctgacggtgcacgaaagctcgctgagtgcctcgattcacgcggtgctggccgccgagctcggtaagcaggataaggccgttgaactctatcagcgtacggctcgtctggacctggacaactacaacaacgatacggcagacggtctgcacatcacctcgatgaccggcggctggctggctatcgtgcagggcttcgccggcatgcgctacgaccacgatcagctgcggttcgatccgttcctgccgaagcagtggcagggttaccagttccgcatcaactaccgcggccgggtgatccaggtcgcggtggggaaaaccgttgcagtgaccctgctggccggcccgccgctgaccgtcatggttgccggccagccgcagcatttggaggtgagcgcgcatgcttaaaggattgctgttcgacctcgacggcgtcttgaccgactcggccaagttccacctgcaggcctggagccagctggccacccagctgggcatcaccctgacgccggccgagcgcgaaggcctgcgcggccgctcgcggctggactcgctgaacctgattttggcggcaggcgcccaggaagaccggttcagtgccgcagagaaaacggcgctaaccgaccagaagaacgcggtgtacctgaagctgattcagacgatgacgccggtggacatcctgccgggcattccgcaactgctgaaggacgcgcaggcggccggcctgaaaatggcaatcgcctcggcgtcgcggaacgccccgacaattcttgaccacctgggcctggccgccagtttcgacgccatcgtcgatccggcgaccctgcaccgcggcaagcccgacccggagatctaccagcaggcgcaagcgctgctggggctccaggccgccgaggtgatcggcttcgaggatgcctcggccggggtcgccgccatcaaagcggccggtcagttcgcggttggcatcggggatgcccggcttctggccgcagcggattacctagtgaaagacacggcggccctgcagctgagccagttgcaagcggcgttcgccaaagaaagtggggagactaatggttgaaatcgacttggaccacctctacaagaagtacgacgacggcgaggattactcggtggtggacttcgaccttcacatcaaggataaggagttcatcgtgttcgtcggcccctcgggctgcgggaagtccaccacgctgcgtatgattgcggggctggaggacattaccaaaggcgagctgaaaatcgacgataaggtgatgaacgacgtggcccccaaggaccgcaacatcgccatggtgtttcagaactacgccttgtacccgcacatgtcagtgtacgacaacatggcgttcggcctaaagctacggcactacaagaaggaggacatcgacaaacgcgtgcaaaacgcggcggagatcctcggcctgaagccgtttctcgaccggaagccggccgccttgtccgggggccagcggcagcgggtggccttgggccgggccatcgtccgcgacgccccaattttcctgatggatgagccgttgtcgaacctggacgcgaagctgcgggtgtccatgcgggcggaaatcgccaagctccaccagcgcctgaacaccaccacgatttacgtgacccacgaccaaaccgaggccatgactatggccgaccgggttgtcgtcatgtccgttggccacgtgcagcagattggcaccccggccgagatttaccagaacccgcggaaccagttcgtggccgggttcatcgggtcgccggcgatgaacttcttcaacatgacctaccaggacggcttcgtcagcgacggccaaagcattcgcctcaaagtgccggaaggccgggcgaagattctggacgaccaagggtacaacggcaaggaagtcgtgttcggcatccggccggaggacatccattcggaggaggccttcctggagacctggccggacgcggttatcagctcaaccgtgtcggtgtcagagctcctgggcgccaccgagcagctttacctgaaggcggatgacaccgagtacgttgccaacgtcaacgcgcgcgacttccacaatcccggggatcatgtgaaaatgggcttcgacgtcaacaaggcgcacttcttcaacaaggacacgaccatggccatcgtggctaagccgattccgctggaaggctgaggaggtgagtgcatgaccccatggtggcagcaagccgtcatttaccagatctacccgaagagttttcaggacagcaacggggatggcatcggcgatttgccggggattaccagtcgccttgattaccttaagcggctgggcgtcgatgccctttggctgagcccagtgtatgtgtcgcccggcgaggacaacggctacgacatcgcggactacgaggccatcgatccccagttcgggacgatggccgacatggacgccttgatcgccgccgccaagcagcgcg

SEQ ID NO: 17 - DNA, 977 bp, Lactobacillus paracasei
cccgcgattttggcgtgattggcttcgacggggtattcctggaccaggtgtccaaccccaagctgaccacggtgaagcagcccgtgcagcgcctcggcgaactgctggcccgcatgctcctgcagaaggtggcacagtccggcgcccaacagggggagctgctggtcgatcctgagctgattgctcgggacacgacgcgaaagtagatcggatttcaactgtccttaccgctatggtagggccagtttttaggctctatgtcaaatctaattcatagctaatagttgatttggcaacgcctaaggcgtcagccatatcttggtaagtatgatggccttcactgaccagttgagctagcgcaccacgttgaaaacgtgataaagtagaagtacccaaagtaatcactccttatagctggttggaattaactactccattgtaagagattgctttgggcctttttttatttttgttcggattaattatagaatttgtctaattagttgaaaattcttagggttgcccatatatcttttagtctggtcattagtttttatgtttgatctgcttttttctgatcgcaaacacccacaactgcgagtgagtcctttttgaagtcgttgactgtcaacaatacatttatttccacattgacattgacagagccaaagcgcgttgccattagaactgcttccaaaaaagctaataactgtgagtcgcccaaacgtttgattagctaaatcgatacgcttttgcatactaatcctcccgcttgataagaaggtacttaaatagttgctttcaattgatctaatcgccattggcaccatgaaataaaggctaattcgtcaatctttggaatgccataggttctagcatacgttaacttttgagtggtgagtagttgatcatagggtttactaataataccaaccacaaggatatcgacttttttgtcaatcccgttgacaggcttt

SEQ ID NO: 18 - DNA, 1239 bp, Lactobacillus paracasei
aaatacgcaaaagaacccgacgagagttaagtctcatcgggttctcagtcgtggatgaattagaagcattgttagctgcataaccttcaacataggatcaatagctggttagatggtcatctctcagactgtttgcaccagatccaggcaaacgtgtttatatccttggtcatactcaggatagatgggcattgtgagtgcaacaggacttagttgcttgtatgctaggcaatgttggccttgatacagaggatcactctgtttctgatctggatgataacctcgtttttccatttcaggacgctgtcccaataattgttgccctgggagtttgtcgaattaagtcttggtgccacaaacacacgctacggcttcttttcttgcaaactgatcttagtatttagggcagttgcatgattacggaattgaaccattttataatgaatcgtcttttctataagtctatagaaagtgcaggtaatggcattttctccagatcggattgtctaatcaatttaattgatttttttggtgtgtttgattatattgcttttgcaaaggtacaatataccttttctctgctgccttgcgagcagcgatggcatcctccatatgaacatatacacgatttaggacaagatggccttgaaagtacagccttgcgacccacttttgagcagttttatcccaactaactccgataacgccagatttgttattggaccgtttaagtgtagaagcaactaaatttgttcgattaattagttgaaaattcttgggattgcccatgtattttttagtctggttattagcttttatgtttgatctgcttatttctgatcgcaaacacccacaactgcgagtgagtcctttttgaagtcgttgactgtcaacgatacatttatttccacattgacattgacagagccaaagcgcgtttccattagaactgcttccaaaaaaactaatgactgtgagtcgtccaaacgtttgattggccaaatcgatacgcttttgcatactaatctccccgtttgataagaaggtacttaaagagttgttttcaattgatctagtcgccattggcaccatgaaataaaggctaattcgtcaatctttggaatgccataggttctagcatacgttaacttttgagtggtaagtagttgatcatagggtttgctaataataccaaccacaaggatatcgacatttttgtcaatcccgttgacaggtttt